European Patent Specification EP 3 850 089 B1, published December 13, 2023. Title: POLYNUCLEOTIDES. Applicant: FREELINE THERAPEUTICS LIMITED. The sequence listing filed with the application follows.

SEQUENCE LISTING (25 sequences)

SEQ ID NO: 1 - DNA, 1494 bp, Artificial Sequence
  Synthetic construct
gccaggccctgcatccctaagagctttggctacagctctgtggtgtgtgtgtgcaatgccacctactgtgacagctttgacccccccacctttcctgccctgggcaccttcagcagatatgagagcaccaggtctgggaggaggatggagctgagcatggggcccatccaggctaatcacactggcactggcctgctgctgaccctgcagcctgagcagaagttccagaaagtaaagggctttggaggggccatgactgatgctgctgctctgaacatcctggccctgagcccccctgcccagaatctgctgctgaagagctacttctctgaggagggcattggctataacatcatcagggtgcccatggccagctgtgacttcagcatcaggacctacacctatgctgacacccctgatgatttccagctgcacaacttcagcctgcctgaggaggataccaagctgaagatcccactgatccacagggctctgcagctggcccagaggcctgtgagcctgctggccagcccctggaccagccccacttggctgaagaccaatggggctgtgaatgggaaggggagcctgaagggacagcctggagacatctaccaccagacctgggccagatactttgtgaagttcctggatgcctatgctgagcacaagctgcagttctgggctgtgactgctgagaatgagccttctgctgggctgctgtctggctaccccttccaatgcctgggcttcacccctgagcatcagagggacttcattgccagggacctgggccctaccctggccaacagcactcaccataatgttaggctgctgatgctggatgaccagaggctgctgctgccccactgggctaaggtggtgctgactgaccctgaggctgctaaatatgtgcatggcattgctgtgcattggtacctggactttctggctcctgccaaggccaccctgggggagacccacaggctgttccccaacaccatgctgtttgcctctgaggcctgtgtgggcagcaagttctgggagcagtctgtgaggctgggcagctgggatagggggatgcagtacagccacagcatcatcaccaacctgctgtaccatgtggtgggctggactgactggaacctggccctgaaccctgagggaggacctaactgggtcagaaactttgtggacagccccatcattgtggacatcaccaaggacaccttttacaagcagcccatgttctaccacctgggccacttcagcaagttcatccctgagggcagccagagagtggggctggtggccagccagaagaatgacctggatgctgtggctctgatgcatcctgatggctctgctgtggtggtggtgctgaacaggagctctaaggatgtgcctctgaccatcaaggatcctgctgtgggcttcctggagaccatcagccctggctacagcatccacacctacctgtggaggaggcagtga

SEQ ID NO: 2 - DNA, 1494 bp, Artificial Sequence
  Synthetic construct
gccaggccctgtatccctaagagctttggctacagctcagtagtttgtgtctgtaatgccacatactgtgactcctttgacccccctaccttccctgccctgggaaccttcagcagatatgagtcaacaagatcaggaaggaggatggagctgtcaatgggacccatccaggctaatcacacaggcacaggcctgctgctgaccctgcagccagaacagaagttccagaaagtgaagggatttggaggagccatgacagatgctgctgctctcaacatcctggccctgtcaccccctgcccagaatctgctgctgaagtcatacttctctgaagaaggaattggatataacatcatcagggtgcccatggccagctgtgacttctccatcaggacctacacctatgctgacacccctgatgatttccagctgcacaacttcagcctcccagaggaagataccaagctcaagatccctctgatacatagggcactgcagctggcccagaggcctgtgtcactcctggccagcccctggacatcacccacttggctcaagaccaatggagctgtgaatggaaagggatcactcaagggacagcctggagacatctaccaccagacctgggccagatactttgtgaagttcctggatgcctatgctgagcacaagctgcagttctgggcagtgacagctgaaaatgagccttctgctggactgctgtcaggataccccttccagtgtctgggcttcacccctgaacatcagagggacttcattgccagggacctgggacctacccttgccaactcaactcaccacaatgtcaggctgctcatgctggatgaccagaggctgctgctgccccactgggccaaggtggtgctgacagacccagaagctgctaaatatgtgcatggcattgctgtgcattggtacctggacttcctggctccagccaaggccaccctgggagagacacacaggctgttccccaacaccatgctctttgcctctgaggcctgtgtgggctccaagttctgggagcagtcagtgaggctgggctcctgggataggggaatgcagtacagccacagcatcatcacaaacctcctgtaccatgtggtgggctggactgactggaacctggccctgaaccctgaaggaggacccaactgggtcagaaattttgtggactcacccatcattgtggacatcaccaaggacacattctacaagcagcccatgttctaccacctgggccacttcagcaagttcatccctgagggctcccagagggtgggactggtggcctcacagaagaatgacctggatgcagtggccctgatgcatcctgatggctctgctgtggtggttgtgctgaatagatcctctaaggatgtgcctctgaccatcaaggatcctgctgtgggcttcctggagacaatctcacctggctactccatccacacctacctgtggaggaggcagtga

SEQ ID NO: 3 - DNA, 1494 bp, Artificial Sequence
  Synthetic construct
gccaggccctgcatccctaagagctttggctacagctctgtggtgtgtgtgtgcaatgccacatactgtgactcctttgacccccccacctttcctgccctgggcacattctccagatatgagagcacaagatctgggagaaggatggagctgagcatggggcccatccaggctaatcacactggcacaggcctgctgctgaccctgcagcctgaacagaagtttcagaaagtgaagggatttggaggggccatgacagatgctgctgctctgaatatcctggccctgtcaccccctgcccagaatctgctgctgaagagctacttttcagaagaaggaattggatataatatcatcagagtgcccatggccagctgtgacttttccatcagaacctacacctatgcagacacccctgatgattttcagctgcacaattttagcctgcctgaggaagataccaagctgaagatacccctgattcacagggccctgcagctggcccagaggcctgtttcactgctggccagcccctggacatcacccacctggctgaagaccaatggagctgtgaatgggaaggggtcactgaagggacagcctggagacatctaccaccagacctgggccagatactttgtgaagtttctggatgcctatgctgagcacaagctgcagttttgggcagtgacagctgaaaatgagccttcagctgggctgctgtcaggatacccctttcagtgcctgggctttacccctgaacatcagagggactttattgccagggacctgggccctaccctggccaatagcacccaccataatgtgaggttgctgatgctggatgaccagaggctgctgctgccccactgggcaaaggtggtgctgacagaccctgaagcagctaaatatgttcatggcattgctgtgcattggtacctggactttctggctcctgccaaggccaccctgggggagacacacaggctgtttcccaataccatgctgtttgcctctgaggcctgtgtgggctccaagttttgggagcagtctgtgaggctgggctcctgggatagagggatgcagtacagccacagcatcatcaccaatctgctgtaccatgtggtgggctggactgactggaatctggccctgaatcctgaaggaggacctaactgggtcaggaattttgtggacagccccatcattgtggacatcaccaaggacaccttttacaagcagcccatgttttaccacctgggccactttagcaagtttattcctgagggctcccagagagtggggctggttgccagccagaagaatgacctggatgcagtggcactgatgcatcctgatggctcagctgttgtggtggtgctgaatagatccagcaaggatgtgcctctgaccatcaaggatcctgctgtgggctttctggagacaatctcacctggctactccattcacacctacctgtggagaaggcagtga

SEQ ID NO: 4 - DNA, 1494 bp, Artificial Sequence
  Synthetic construct
gccaggccttgcatcccaaagtctttcggctacagctccgtggtgtgcgtgtgcaacgccacctattgtgactccttcgatccccctacctttcccgccctgggcacattttctagatacgagtctacacgcagcggccggagaatggagctgagcatgggccctatccaggccaatcacacaggaacaggcctgctgctgaccctgcagccagagcagaagttccagaaggtgaagggctttggcggagccatgacagatgcagccgccctgaacatcctggccctgtccccacccgcccagaatctgctgctgaagtcctacttctctgaggagggcatcggctataacatcatccgggtgcccatggccagctgcgacttttccatcagaacctacacatatgccgatacccctgacgatttccagctgcacaatttttccctgccagaggaggatacaaagctgaagatccccctgattcaccgggccctgcagctggcacagcggcccgtgagcctgctggccagcccctggacctcccctacatggctgaagaccaacggcgccgtgaatggcaagggctctctgaagggacagcctggcgacatctaccaccagacatgggccagatatttcgtgaagtttctggatgcctacgccgagcacaagctgcagttctgggccgtgacagcagagaatgagccttctgccggcctgctgagcggctatcccttccagtgcctgggctttacacctgagcaccagcgggactttatcgccagagatctgggcccaaccctggccaactccacacaccacaatgtgaggctgctgatgctggacgatcagcgcctgctgctgcctcactgggccaaggtggtgctgaccgacccagaggccgccaagtacgtgcacggcatcgccgtgcactggtatctggatttcctggcacctgcaaaggccaccctgggagagacacaccggctgttccctaacaccatgctgtttgccagcgaggcctgcgtgggctccaagttttgggagcagtccgtgaggctgggatcttgggacagaggcatgcagtactcccactctatcatcaccaatctgctgtatcacgtggtgggctggacagactggaacctggccctgaatccagagggcggccccaactgggtgagaaatttcgtggatagccccatcatcgtggacatcaccaaggatacattctacaagcagccaatgttttatcacctgggccacttctctaagtttatccctgagggcagccagagggtgggcctggtggccagccagaagaacgacctggatgccgtggccctgatgcaccctgatggctccgccgtggtggtggtgctgaatcgctctagcaaggacgtgcctctgaccatcaaggatccagccgtgggatttctggagactatttcacctggctattcaattcatacctacctgtggaggaggcagtga

SEQ ID NO: 5 - DNA, 1611 bp, Artificial Sequence
  Synthetic construct
atggagttttcaagtccttccagagaggaatgtcccaagcctttgagtagggtaagcatcatggctggcagcctcacaggattgcttctacttcaggcagtgtcgtgggcatcaggtgccaggccctgcatccctaagagctttggctacagctctgtggtgtgtgtgtgcaatgccacctactgtgacagctttgacccccccacctttcctgccctgggcaccttcagcagatatgagagcaccaggtctgggaggaggatggagctgagcatggggcccatccaggctaatcacactggcactggcctgctgctgaccctgcagcctgagcagaagttccagaaagtaaagggctttggaggggccatgactgatgctgctgctctgaacatcctggccctgagcccccctgcccagaatctgctgctgaagagctacttctctgaggagggcattggctataacatcatcagggtgcccatggccagctgtgacttcagcatcaggacctacacctatgctgacacccctgatgatttccagctgcacaacttcagcctgcctgaggaggataccaagctgaagatcccactgatccacagggctctgcagctggcccagaggcctgtgagcctgctggccagcccctggaccagccccacttggctgaagaccaatggggctgtgaatgggaaggggagcctgaagggacagcctggagacatctaccaccagacctgggccagatactttgtgaagttcctggatgcctatgctgagcacaagctgcagttctgggctgtgactgctgagaatgagccttctgctgggctgctgtctggctaccccttccaatgcctgggcttcacccctgagcatcagagggacttcattgccagggacctgggccctaccctggccaacagcactcaccataatgttaggctgctgatgctggatgaccagaggctgctgctgccccactgggctaaggtggtgctgactgaccctgaggctgctaaatatgtgcatggcattgctgtgcattggtacctggactttctggctcctgccaaggccaccctgggggagacccacaggctgttccccaacaccatgctgtttgcctctgaggcctgtgtgggcagcaagttctgggagcagtctgtgaggctgggcagctgggatagggggatgcagtacagccacagcatcatcaccaacctgctgtaccatgtggtgggctggactgactggaacctggccctgaaccctgagggaggacctaactgggtcagaaactttgtggacagccccatcattgtggacatcaccaaggacaccttttacaagcagcccatgttctaccacctgggccacttcagcaagttcatccctgagggcagccagagagtggggctggtggccagccagaagaatgacctggatgctgtggctctgatgcatcctgatggctctgctgtggtggtggtgctgaacaggagctctaaggatgtgcctctgaccatcaaggatcctgctgtgggcttcctggagaccatcagccctggctacagcatccacacctacctgtggaggaggcagtga

SEQ ID NO: 6 - DNA, 1611 bp, Artificial Sequence
  Synthetic construct
atggagttttcaagtccttccagagaggaatgtcccaagcctttgagtagggtaagcatcatggctggcagcctcacaggattgcttctacttcaggcagtgtcgtgggcatcaggtgccaggccctgtatccctaagagctttggctacagctcagtagtttgtgtctgtaatgccacatactgtgactcctttgacccccctaccttccctgccctgggaaccttcagcagatatgagtcaacaagatcaggaaggaggatggagctgtcaatgggacccatccaggctaatcacacaggcacaggcctgctgctgaccctgcagccagaacagaagttccagaaagtgaagggatttggaggagccatgacagatgctgctgctctcaacatcctggccctgtcaccccctgcccagaatctgctgctgaagtcatacttctctgaagaaggaattggatataacatcatcagggtgcccatggccagctgtgacttctccatcaggacctacacctatgctgacacccctgatgatttccagctgcacaacttcagcctcccagaggaagataccaagctcaagatccctctgatacatagggcactgcagctggcccagaggcctgtgtcactcctggccagcccctggacatcacccacttggctcaagaccaatggagctgtgaatggaaagggatcactcaagggacagcctggagacatctaccaccagacctgggccagatactttgtgaagttcctggatgcctatgctgagcacaagctgcagttctgggcagtgacagctgaaaatgagccttctgctggactgctgtcaggataccccttccagtgtctgggcttcacccctgaacatcagagggacttcattgccagggacctgggacctacccttgccaactcaactcaccacaatgtcaggctgctcatgctggatgaccagaggctgctgctgccccactgggccaaggtggtgctgacagacccagaagctgctaaatatgtgcatggcattgctgtgcattggtacctggacttcctggctccagccaaggccaccctgggagagacacacaggctgttccccaacaccatgctctttgcctctgaggcctgtgtgggctccaagttctgggagcagtcagtgaggctgggctcctgggataggggaatgcagtacagccacagcatcatcacaaacctcctgtaccatgtggtgggctggactgactggaacctggccctgaaccctgaaggaggacccaactgggtcagaaattttgtggactcacccatcattgtggacatcaccaaggacacattctacaagcagcccatgttctaccacctgggccacttcagcaagttcatccctgagggctcccagagggtgggactggtggcctcacagaagaatgacctggatgcagtggccctgatgcatcctgatggctctgctgtggtggttgtgctgaatagatcctctaaggatgtgcctctgaccatcaaggatcctgctgtgggcttcctggagacaatctcacctggctactccatccacacctacctgtggaggaggcagtga

SEQ ID NO: 7 - DNA, 1611 bp, Artificial Sequence
  Synthetic construct
atggagttttcaagtccttccagagaggaatgtcccaagcctttgagtagggtaagcatcatggctggcagcctcacaggattgcttctacttcaggcagtgtcgtgggcatcaggtgccaggccctgcatccctaagagctttggctacagctctgtggtgtgtgtgtgcaatgccacatactgtgactcctttgacccccccacctttcctgccctgggcacattctccagatatgagagcacaagatctgggagaaggatggagctgagcatggggcccatccaggctaatcacactggcacaggcctgctgctgaccctgcagcctgaacagaagtttcagaaagtgaagggatttggaggggccatgacagatgctgctgctctgaatatcctggccctgtcaccccctgcccagaatctgctgctgaagagctacttttcagaagaaggaattggatataatatcatcagagtgcccatggccagctgtgacttttccatcagaacctacacctatgcagacacccctgatgattttcagctgcacaattttagcctgcctgaggaagataccaagctgaagatacccctgattcacagggccctgcagctggcccagaggcctgtttcactgctggccagcccctggacatcacccacctggctgaagaccaatggagctgtgaatgggaaggggtcactgaagggacagcctggagacatctaccaccagacctgggccagatactttgtgaagtttctggatgcctatgctgagcacaagctgcagttttgggcagtgacagctgaaaatgagccttcagctgggctgctgtcaggatacccctttcagtgcctgggctttacccctgaacatcagagggactttattgccagggacctgggccctaccctggccaatagcacccaccataatgtgaggttgctgatgctggatgaccagaggctgctgctgccccactgggcaaaggtggtgctgacagaccctgaagcagctaaatatgttcatggcattgctgtgcattggtacctggactttctggctcctgccaaggccaccctgggggagacacacaggctgtttcccaataccatgctgtttgcctctgaggcctgtgtgggctccaagttttgggagcagtctgtgaggctgggctcctgggatagagggatgcagtacagccacagcatcatcaccaatctgctgtaccatgtggtgggctggactgactggaatctggccctgaatcctgaaggaggacctaactgggtcaggaattttgtggacagccccatcattgtggacatcaccaaggacaccttttacaagcagcccatgttttaccacctgggccactttagcaagtttattcctgagggctcccagagagtggggctggttgccagccagaagaatgacctggatgcagtggcactgatgcatcctgatggctcagctgttgtggtggtgctgaatagatccagcaaggatgtgcctctgaccatcaaggatcctgctgtgggctttctggagacaatctcacctggctactccattcacacctacctgtggagaaggcagtga

SEQ ID NO: 8 - DNA, 1611 bp, Artificial Sequence
  Synthetic construct
atggagttttcaagtccttccagagaggaatgtcccaagcctttgagtagggtaagcatcatggctggcagcctcacaggattgcttctacttcaggcagtgtcgtgggcatcaggtgccaggccttgcatcccaaagtctttcggctacagctccgtggtgtgcgtgtgcaacgccacctattgtgactccttcgatccccctacctttcccgccctgggcacattttctagatacgagtctacacgcagcggccggagaatggagctgagcatgggccctatccaggccaatcacacaggaacaggcctgctgctgaccctgcagccagagcagaagttccagaaggtgaagggctttggcggagccatgacagatgcagccgccctgaacatcctggccctgtccccacccgcccagaatctgctgctgaagtcctacttctctgaggagggcatcggctataacatcatccgggtgcccatggccagctgcgacttttccatcagaacctacacatatgccgatacccctgacgatttccagctgcacaatttttccctgccagaggaggatacaaagctgaagatccccctgattcaccgggccctgcagctggcacagcggcccgtgagcctgctggccagcccctggacctcccctacatggctgaagaccaacggcgccgtgaatggcaagggctctctgaagggacagcctggcgacatctaccaccagacatgggccagatatttcgtgaagtttctggatgcctacgccgagcacaagctgcagttctgggccgtgacagcagagaatgagccttctgccggcctgctgagcggctatcccttccagtgcctgggctttacacctgagcaccagcgggactttatcgccagagatctgggcccaaccctggccaactccacacaccacaatgtgaggctgctgatgctggacgatcagcgcctgctgctgcctcactgggccaaggtggtgctgaccgacccagaggccgccaagtacgtgcacggcatcgccgtgcactggtatctggatttcctggcacctgcaaaggccaccctgggagagacacaccggctgttccctaacaccatgctgtttgccagcgaggcctgcgtgggctccaagttttgggagcagtccgtgaggctgggatcttgggacagaggcatgcagtactcccactctatcatcaccaatctgctgtatcacgtggtgggctggacagactggaacctggccctgaatccagagggcggccccaactgggtgagaaatttcgtggatagccccatcatcgtggacatcaccaaggatacattctacaagcagccaatgttttatcacctgggccacttctctaagtttatccctgagggcagccagagggtgggcctggtggccagccagaagaacgacctggatgccgtggccctgatgcaccctgatggctccgccgtggtggtggtgctgaatcgctctagcaaggacgtgcctctgaccatcaaggatccagccgtgggatttctggagactatttcacctggctattcaattcatacctacctgtggaggaggcagtga

SEQ ID NO: 9 - DNA, 1611 bp, Homo sapiens
atggagttttcaagtccttccagagaggaatgtcccaagcctttgagtagggtaagcatcatggctggcagcctcacaggattgcttctacttcaggcagtgtcgtgggcatcaggtgcccgcccctgcatccctaaaagcttcggctacagctcggtggtgtgtgtctgcaatgccacatactgtgactcctttgaccccccgacctttcctgcccttggtaccttcagccgctatgagagtacacgcagtgggcgacggatggagctgagtatggggcccatccaggctaatcacacgggcacaggcctgctactgaccctgcagccagaacagaagttccagaaagtgaagggatttggaggggccatgacagatgctgctgctctcaacatccttgccctgtcaccccctgcccaaaatttgctacttaaatcgtacttctctgaagaaggaatcggatataacatcatccgggtacccatggccagctgtgacttctccatccgcacctacacctatgcagacacccctgatgatttccagttgcacaacttcagcctcccagaggaagataccaagctcaagatacccctgattcaccgagccctgcagttggcccagcgtcccgtttcactccttgccagcccctggacatcacccacttggctcaagaccaatggagcggtgaatgggaaggggtcactcaagggacagcccggagacatctaccaccagacctgggccagatactttgtgaagttcctggatgcctatgctgagcacaagttacagttctgggcagtgacagctgaaaatgagccttctgctgggctgttgagtggataccccttccagtgcctgggcttcacccctgaacatcagcgagacttcattgcccgtgacctaggtcctaccctcgccaacagtactcaccacaatgtccgcctactcatgctggatgaccaacgcttgctgctgccccactgggcaaaggtggtactgacagacccagaagcagctaaatatgttcatggcattgctgtacattggtacctggactttctggctccagccaaagccaccctaggggagacacaccgcctgttccccaacaccatgctctttgcctcagaggcctgtgtgggctccaagttctgggagcagagtgtgcggctaggctcctgggatcgagggatgcagtacagccacagcatcatcacgaacctcctgtaccatgtggtcggctggaccgactggaaccttgccctgaaccccgaaggaggacccaattgggtgcgtaactttgtcgacagtcccatcattgtagacatcaccaaggacacgttttacaaacagcccatgttctaccaccttggccacttcagcaagttcattcctgagggctcccagagagtggggctggttgccagtcagaagaacgacctggacgcagtggcactgatgcatcccgatggctctgctgttgtggtcgtgctaaaccgctcctctaaggatgtgcctcttaccatcaaggatcctgctgtgggcttcctggagacaatctcacctggctactccattcacacctacctgtggcgtcgccagtga

SEQ ID NO: 10 - DNA, 334 bp, Artificial Sequence
  Synthetic construct
ccctaaaatgggcaaacattgcaagcagcaaacagcaaacacacagccctccctgcctgctgaccttggagctggggcagaggtcagacacctctctgggcccatgccacctccaactggacacaggacgctgtggtttctgagccagggggcgactcagatcccagccagtggacttagcccctgtttgctcctccgataactggggtgaccttggttaatattcaccagcagcctcccccgttgcccctctggatccactgcttaaatacggacgaggacagggccctgtctcctcagcttcaggcaccaccactgacctgggacagtgaat

SEQ ID NO: 11 - DNA, 117 bp, Artificial Sequence
  Synthetic construct
ccctaaaatgggcaaacattgcaagcagcaaacagcaaacacacagccctccctgcctgctgaccttggagctggggcagaggtcagacacctctctgggcccatgccacctccaac

SEQ ID NO: 12 - DNA, 185 bp, Artificial Sequence
  Synthetic construct
gggcgactcagatcccagccagtggacttagcccctgtttgctcctccgataactggggtgaccttggttaatattcaccagcagcctcccccgttgcccctctggatccactgcttaaatacggacgaggacagggccctgtctcctcagcttcaggcaccaccactgacctgggacagtgaat

SEQ ID NO: 13 - DNA, 659 bp, Artificial Sequence
  Synthetic construct
gacattgattattgactagttattaatagtaatcaattacggggtcattagttcatagcccatatatggagttccgcgttacataacttacggtaaatggcccgcctggctgaccgcccaacgacccccgcccattgacgtcaataatgacgtatgttcccatagtaacgccaatagggactttccattgacgtcaatgggtggagtatttacggtaaactgcccacttggcagtacatcaagtgtatcatatgccaagtacgccccctattgacgtcaatgacggtaaatggcccgcctggcattatgcccagtacatgaccttatgggactttcctacttggcagtacatctacgtattagtcatcgctattaccatggtcgaggtgagccccacgttctgcttcactctccccatctcccccccctccccacccccaattttgtatttatttattttttaattattttgtgcagcgatgggggcggggggggggggggggcgcgcgccaggcggggcggggcggggcgaggggcggggcggggcgaggcggagaggtgcggcggcagccaatcagagcggcgcgctccgaaagtttccttttatggcgaggcggcggcggcggcggccctataaaaagcgaagcgcgcggcgggcg

SEQ ID NO: 14 - DNA, 747 bp, Artificial Sequence
  Synthetic construct
aggctcagaggcacacaggagtttctgggctcaccctgcccccttccaacccctcagttcccatcctccagcagctgtttgtgtgctgcctctgaagtccacactgaacaaacttcagcctactcatgtccctaaaatgggcaaacattgcaagcagcaaacagcaaacacacagccctccctgcctgctgaccttggagctggggcagaggtcagagacctctctgggcccatgccacctccaacatccactcgaccccttggaatttcggtggagaggagcagaggttgtcctggcgtggtttaggtagtgtgagaggggtacccggggatcttgctaccagtggaacagccactaaggattctgcagtgagagcagagggccagctaagtggtactctcccagagactgtctgactcacgccaccccctccaccttggacacaggacgctgtggtttctgagccaggtacaatgactcctttcggtaagtgcagtggaagctgtacactgcccaggcaaagcgtccgggcagcgtaggcgggcgactcagatcccagccagtggacttagcccctgtttgctcctccgataactggggtgaccttggttaatattcaccagcagcctcccccgttgcccctctggatccactgcttaaatacggacgaggacagggccctgtctcctcagcttcaggcaccaccactgacctgggacagtgaatgatccccctgatctgcggcc

SEQ ID NO: 15 - DNA, 418 bp, Artificial Sequence
  Synthetic construct
ggatcttgctaccagtggaacagccactaaggattctgcagtgagagcagagggccagctaagtggtactctcccagagactgtctgactcacgccaccccctccaccttggacacaggacgctgtggtttctgagccaggtacaatgactcctttcggtaagtgcagtggaagctgtacactgcccaggcaaagcgtccgggcagcgtaggcgggcgactcagatcccagccagtggacttagcccctgtttgctcctccgataactggggtgaccttggttaatattcaccagcagcctcccccgttgcccctctggatccactgcttaaatacggacgaggacagggccctgtctcctcagcttcaggcaccaccactgacctgggacagtgaatgatccccctgatctgcggcc

SEQ ID NO: 16 - DNA, 321 bp, Artificial Sequence
  Synthetic construct
aggctcagaggcacacaggagtttctgggctcaccctgcccccttccaacccctcagttcccatcctccagcagctgtttgtgtgctgcctctgaagtccacactgaacaaacttcagcctactcatgtccctaaaatgggcaaacattgcaagcagcaaacagcaaacacacagccctccctgcctgctgaccttggagctggggcagaggtcagagacctctctgggcccatgccacctccaacatccactcgaccccttggaatttcggtggagaggagcagaggttgtcctggcgtggtttaggtagtgtgagaggg

SEQ ID NO: 17 - DNA, 117 bp, Homo sapiens
atggagttttcaagtccttccagagaggaatgtcccaagcctttgagtagggtaagcatcatggctggcagcctcacaggattgcttctacttcaggcagtgtcgtgggcatcaggt

SEQ ID NO: 18 - protein, 39 aa, Homo sapiens
MEFSSPSREECPKPLSRVSIMAGSLTGLLLLQAVSWASG

SEQ ID NO: 19 - protein, 736 aa, adeno-associated virus 3B
MAADGYLPDWLEDNLSEGIREWWALKPGVPQPKANQQHQDNRRGLVLPGYKYLGPGNGLDKGEPVNEADAAALEHDKAYDQQLKAGDNPYLKYNHADAEFQERLQEDTSFGGNLGRAVFQAKKRILEPLGLVEEAAKTAPGKKRPVDQSPQEPDSSSGVGKSGKQPARKRLNFGQTGDSESVPDPQPLGEPPAAPTSLGSNTMASGGGAPMADNNEGADGVGNSSGNWHCDSQWLGDRVITTSTRTWALPTYNNHLYKQISSQSGASNDNHYFGYSTPWGYFDFNRFHCHFSPRDWQRLINNNWGFRPKKLSFKLFNIQVKEVTQNDGTTTIANNLTSTVQVFTDSEYQLPYVLGSAHQGCLPPFPADVFMVPQYGYLTLNNGSQAVGRSSFYCLEYFPSQMLRTGNNFQFSYTFEDVPFHSSYAHSQSLDRLMNPLIDQYLYYLNRTQGTTSGTTNQSRLLFSQAGPQSMSLQARNWLPGPCYRQQRLSKTANDNNNSNFPWTAASKYHLNGRDSLVNPGPAMASHKDDEEKFFPMHGNLIFGKEGTTASNAELDNVMITDEEEIRTTNPVATEQYGTVANNLQSSNTAPTTRTVNDQGALPGMVWQDRDVYLQGPIWAKIPHTDGHFHPSPLMGGFGLKHPPPQIMIKNTPVPANPPTTFSPAKFASFITQYSTGQVSVEIEWELQKENSKRWNPEIQYTSNYNKSVNVDFTVDTNGVYSEPRPIGTRYLTRNL

SEQ ID NO: 20 - protein, 736 aa, Artificial Sequence
  Synthetic capsid protein
MAADGYLPDWLEDNLSEGIREWWALKPGAPKPKANQQKQDDGRGLVLPGYKYLGPFNGLDKGEPVNAADAAALEHDKAYDQQLQAGDNPYLRYNHADAEFQERLQEDTSFGGNLGRAVFQAKKRVLEPLGLVEEGAKTAPGKKRPVDQSPQEPDSSSGVGKSGKQPARKRLNFGQTGDSESVPDPQPLGEPPAAPTSLGSNTMASGGGAPMADNNEGADGVGNSSGNWHCDSQWLGDRVITTSTRTWALPTYNNHLYKQISSQSGASNDNHYFGYSTPWGYFDFNRFHCHFSPRDWQRLINNNWGFRPKKLSFKLFNIQVKEVTQNDGTTTIANNLTSTVQVFTDSEYQLPYVLGSAHQGCLPPFPADVFMVPQYGYLTLNNGSQAVGRSSFYCLEYFPSQMLRTGNNFQFSYTFEDVPFHSSYAHSQSLDRLMNPLIDQYLYYLNRTQGTTSGTTNQSRLLFSQAGPQSMSLQARNWLPGPCYRQQRLSKTANDNNNSNFPWTAASKYHLNGRDSLVNPGPAMASHKDDEEKFFPMHGNLIFGKEGTTASNAELDNVMITDEEEIRTTNPVATEQYGTVANNLQSSNTAPTTRTVNDQGALPGMVWQDRDVYLQGPIWAKIPHTDGHFHPSPLMGGFGLKHPPPQIMIKNTPVPANPPTTFSPAKFASFITQYSTGQVSVEIEWELQKENSKRWNPEIQYTSNYNKSVNVDFTVDTNGVYSEPRPIGTRYLTRNL

SEQ ID NO: 21 - protein, 736 aa, adeno-associated virus 9
MAADGYLPDWLEDNLSEGIREWWALKPGAPQPKANQQHQDNARGLVLPGYKYLGPGNGLDKGEPVNAADAAALEHDKAYDQQLKAGDNPYLKYNHADAEFQERLKEDTSFGGNLGRAVFQAKKRLLEPLGLVEEAAKTAPGKKRPVEQSPQEPDSSAGIGKSGAQPAKKRLNFGQTGDTESVPDPQPIGEPPAAPSGVGSLTMASGGGAPVADNNEGADGVGSSSGNWHCDSQWLGDRVITTSTRTWALPTYNNHLYKQISNSTSGGSSNDNAYFGYSTPWGYFDFNRFHCHFSPRDWQRLINNNWGFRPKRLNFKLFNIQVKEVTDNNGVKTIANNLTSTVQVFTDSDYQLPYVLGSAHEGCLPPFPADVFMIPQYGYLTLNDGSQAVGRSSFYCLEYFPSQMLRTGNNFQFSYEFENVPFHSSYAHSQSLDRLMNPLIDQYLYYLSKTINGSGQNQQTLKFSVAGPSNMAVQGRNYIPGPSYRQQRVSTTVTQNNNSEFAWPGASSWALNGRNSLMNPGPAMASHKEGEDRFFPLSGSLIFGKQGTGRDNVDADKVMITNEEEIKTTNPVATESYGQVATNHQSAQAQAQTGWVQNQGILPGMVWQDRDVYLQGPIWAKIPHTDGNFHPSPLMGGFGMKHPPPQILIKNTPVPADPPTAFNKDKLNSFITQYSTGQVSVEIEWELQKENSKRWNPEIQYTSNYYKSNNVEFAVNTEGVYSEPRPIGTRYLTRNL

SEQ ID NO: 22 - DNA, 66 bp, Simian virus 40
gtaaatataaaatttttaagtgtataatgtgttaaactactgattctaattgtttctctcttttag

SEQ ID NO: 23 - DNA, 208 bp, Bos taurus
ctgtgccttctagttgccagccatctgttgtttgcccctcccccgtgccttccttgaccctggaaggtgccactcccactgtcctttcctaataaaatgaggaaattgcatcgcattgtctgagtaggtgtcattctattctggggggtggggtggggcaggacagcaagggggaggattgggaagacaatagcaggcatgctgggga

SEQ ID NO: 24 - protein, 736 aa, Artificial Sequence
  Synthetic capsid protein
MAADGYLPDWLEDNLSEGIREWWALQPGAPKPKANQQHQDNARGLVLPGYKYLGPGNGLDKGEPVNAADAAALEHDKAYDQQLKAGDNPYLKYNHADAEFQERLKEDTSFGGNLGRAVFQAKKRLLEPLGLVEEAAKTAPGKKRPVDQSPQEPDSSSGVGKSGKQPARKRLNFGQTGDSESVPDPQPLGEPPAAPTSLGSNTMASGGGAPMADNNEGADGVGNSSGNWHCDSQWLGDRVITTSTRTWALPTYNNHLYKQISSQSGASNDNHYFGYSTPWGYFDFNRFHCHFSPRDWQRLINNNWGFRPKKLSFKLFNIQVKEVTQNDGTTTIANNLTSTVQVFTDSEYQLPYVLGSAHQGCLPPFPADVFMVPQYGYLTLNNGSQAVGRSSFYCLEYFPSQMLRTGNNFQFSYTFEDVPFHSSYAHSQSLDRLMNPLIDQYLYYLNRTQGTTSGTTNQSRLLFSQAGPQSMSLQARNWLPGPCYRQQRLSKTANDNNNSNFPWTAASKYHLNGRDSLVNPGPAMASHKDDEEKFFPMHGNLIFGKEGTTASNAELDNVMITDEEEIRTTNPVATEQYGTVANNLQSSNTAPTTRTVNDQGALPGMVWQDRDVYLQGPIWAKIPHTDGHFHPSPLMGGFGLKHPPPQIMIKNTPVPANPPTTFSPAKFASFITQYSTGQVSVEIEWELQKENSKRWNPEIQYTSNYNKSVNVDFTVDTNGVYSEPRPIGTRYLTRPL

SEQ ID NO: 25 - protein, 536 aa, Homo sapiens
MEFSSPSREECPKPLSRVSIMAGSLTGLLLLQAVSWASGARPCIPKSFGYSSVVCVCNATYCDSFDPPTFPALGTFSRYESTRSGRRMELSMGPIQANHTGTGLLLTLQPEQKFQKVKGFGGAMTDAAALNILALSPPAQNLLLKSYFSEEGIGYNIIRVPMASCDFSIRTYTYADTPDDFQLHNFSLPEEDTKLKIPLIHRALQLAQRPVSLLASPWTSPTWLKTNGAVNGKGSLKGQPGDIYHQTWARYFVKFLDAYAEHKLQFWAVTAENEPSAGLLSGYPFQCLGFTPEHQRDFIARDLGPTLANSTHHNVRLLMLDDQRLLLPHWAKVVLTDPEAAKYVHGIAVHWYLDFLAPAKATLGETHRLFPNTMLFASEACVGSKFWEQSVRLGSWDRGMQYSHSIITNLLYHVVGWTDWNLALNPEGGPNWVRNFVDSPIIVDITKDTFYKQPMFYHLGHFSKFIPEGSQRVGLVASQKNDLDAVALMHPDGSAVVVVLNRSSKDVPLTIKDPAVGFLETISPGYSIHTYLWRRQ